European Patent Application EP 4 137 138 A1, published February 22, 2023. Title: METHODS OF TREATING TRANSTHYRETIN (TTR) MEDIATED AMYLOIDOSIS. Applicant: ALNYLAM PHARMACEUTICALS, INC. The sequence listing filed with the application follows.

SEQUENCE LISTING (5 sequences)

SEQ ID NO: 1 - DNA, 21 bp, Artificial Sequence
  Description of Artificial Sequence: Synthetic oligonucleotide
  Description of Combined DNA/RNA Molecule: Synthetic oligonucleotide
guaaccaagaguauuccautt

SEQ ID NO: 2 - DNA, 21 bp, Artificial Sequence
  Description of Artificial Sequence: Synthetic oligonucleotide
  Description of Combined DNA/RNA Molecule: Synthetic oligonucleotide
auggaauacucuugguuactt

SEQ ID NO: 3 - DNA, 37 bp, Artificial Sequence
  Description of Artificial Sequence: Synthetic primer
aatcaagttaaagtggaatgaaaagtgcctttcacag

SEQ ID NO: 4 - DNA, 30 bp, Artificial Sequence
  Description of Artificial Sequence: Synthetic primer
gcctttcacaggaatgttttattgtctctg

SEQ ID NO: 5 - DNA, 34 bp, Artificial Sequence
  Description of Artificial Sequence: Synthetic primer
ctctgcctggacttctaacatagcatatgaggtg